European Patent Application EP 4 755 907 A2, published June 10, 2026. Title: PHARMACEUTICAL COMPOSITIONS OF HUMANIZED ANTI-CD40 ANTIBODIES AND USES THEREOF. Applicant: Kiniksa Pharmaceuticals, Ltd. Application EP. The sequence listing filed with the application follows.

SEQUENCE LISTING (21 sequences)

SEQ ID NO: 1 - protein, 114 aa, Mus musculus
QVQLQQSGAELAKPGASVKMSCKASGYTFTNYWMHWVKQRPGQGLEWIGYINPSNDYTKYNQKFKDKATLTADKSSNTAYMQLGSLTSEDSAVYYCARQGFPYWGQGTLVTVSA

SEQ ID NO: 2 - protein, 106 aa, Mus musculus
QIVLTQSPAIMSASPGEKVTMTCSASSSVSYMHWYHQRSGTSPKRWIYDTSKLASGVPARFSGSGSGTSYSLTISSMEAEDAATYYCHQLSSDPFTFGSGTKLEIK

SEQ ID NO: 3 - protein, 9 aa, Mus musculus
YTFTNYWMH

SEQ ID NO: 4 - protein, 17 aa, Mus musculus
YINPSNDYTKYNQKFKD

SEQ ID NO: 5 - protein, 5 aa, Mus musculus
QGFPY

SEQ ID NO: 6 - protein, 10 aa, Mus musculus
SASSSVSYMH

SEQ ID NO: 7 - protein, 7 aa, Mus musculus
DTSKLAS

SEQ ID NO: 8 - protein, 9 aa, Mus musculus
HQLSSDPFT

SEQ ID NO: 9 - protein, 114 aa, synthetic construct
QVQLVQSGAEVKKPGASVKVSCKASGYTFTNYWMHWVRQAPGQRLEWIGYINPSNDYTKYNQKFKDRATLTADKSANTAYMELSSLRSEDTAVYYCARQGFPYWGQGTLVTVSS

SEQ ID NO: 10 - protein, 106 aa, synthetic construct
EIVLTQSPATLSLSPGERATLSCSASSSVSYMHWYQQKPGQAPRRWIYDTSKLASGVPARFSGSGSGTDYTLTISSLEPEDFAVYYCHQLSSDPFTFGGGTKVEIK

SEQ ID NO: 11 - protein, 441 aa, synthetic construct
QVQLVQSGAEVKKPGASVKVSCKASGYTFTNYWMHWVRQAPGQRLEWIGYINPSNDYTKYNQKFKDRATLTADKSANTAYMELSSLRSEDTAVYYCARQGFPYWGQGTLVTVSSASTKGPSVFPLAPCSRSTSESTAALGCLVKDYFPEPVTVSWNSGALTSGVHTFPAVLQSSGLYSLSSVVTVPSSSLGTKTYTCNVDHKPSNTKVDKRVESKYGPPCPPCPAPEFLGGPSVFLFPPKPKDTLMISRTPEVTCVVVDVSQEDPEVQFNWYVDGVEVHNAKTKPREEQFNSTYRVVSVLTVLHQDWLNGKEYKCKVSNKGLPSSIEKTISKAKGQPREPQVYTLPPSQEEMTKNQVSLTCLVKGFYPSDIAVEWESNGQPENNYKTTPPVLDSDGSFFLYSRLTVDKSRWQEGNVFSCSVMHEALHNHYTQKSLSLSPGK

SEQ ID NO: 12 - protein, 213 aa, synthetic construct
EIVLTQSPATLSLSPGERATLSCSASSSVSYMHWYQQKPGQAPRRWIYDTSKLASGVPARFSGSGSGTDYTLTISSLEPEDFAVYYCHQLSSDPFTFGGGTKVEIKRTVAAPSVFIFPPSDEQLKSGTASVVCLLNNFYPREAKVQWKVDNALQSGNSQESVTEQDSKDSTYSLSSTLTLSKADYEKHKVYACEVTHQGLSSPVTKSFNRGEC

SEQ ID NO: 13 - protein, 114 aa, Homo sapiens
QVQLVQSGAEVKKPGASVKVSCKASGYTFTNYWMHWVRQAPGQRLEWMGYINPSNDYTKYNQKFKDRVTITRDTSASTAYMELSSLRSEDTAVYYCARQGFPYWGQGTLVTVSS

SEQ ID NO: 14 - protein, 114 aa, Homo sapiens
QVQLVQSGAEVKKPGASVKVSCKASGYTFTNYWMHWVRQAPGQRLEWMGYINPSNDYTKYNQKFKDRVTITADKSASTAYMELSSLRSEDTAVYYCARQGFPYWGQGTLVTVSS

SEQ ID NO: 15 - protein, 106 aa, Homo sapiens
EIVLTQSPATLSLSPGERATLSCSASSSVSYMHWYQQKPGQAPRLLIYDTSKLASGIPARFSGSGSGTDFTLTISSLEPEDFAVYYCHQLSSDPFTFGGGTKVEIK

SEQ ID NO: 16 - protein, 114 aa, Homo sapiens; identical to SEQ ID NO: 9

SEQ ID NO: 17 - protein, 114 aa, Homo sapiens
QVQLVQSGAEVKKPGASVKVSCKASGYTFTNYWMHWVRQAPGQRLEWIGYINPSNDYTKYNQKFKDRATLTADTSTNTAYMELSSLRSEDTAVYYCARQGFPYWGQGTLVTVSS

SEQ ID NO: 18 - protein, 114 aa, Homo sapiens
QVQLVQSGAEVKKPGSSVKVSCKASGYTFTNYWMHWVRQAPGQGLEWIGYINPSNDYTKYNQKFKDKATITADESTNTAYMELSSLRSEDTAVYYCARQGFPYWGQGTLVTVSS

SEQ ID NO: 19 - protein, 106 aa, Homo sapiens; identical to SEQ ID NO: 10

SEQ ID NO: 20 - protein, 106 aa, Homo sapiens
DIQMTQSPSTLSASVGDRVTITCSASSSVSYMHWYQQKPGKAPKLLIYDTSKLASGVPARFSGSGSGTEFTLTISSLQPDDFATYYCHQLSSDPFTFGQGTKVEVK

SEQ ID NO: 21 - protein, 106 aa, Homo sapiens
EIVLTQSPATLSLSPGERATLSCSASSSVSYMHWYQQKPGQAPRLLIYDTSKLASGIPARFSGSGSGTDFTLTISSLEPEDFAVYYCHQLSSDPFTFGQGTKLEIK